European Patent Application EP 4 682 257 A1, published January 21, 2026. Title: Polynucleotide. Applicant: 住友化学株式会社. The sequence listing filed with the application follows.

SEQUENCE LISTING (15 sequences)

SEQ ID NO: 1 - DNA, 1333 bp, Polypedilum vanderplanki
  source 1..1333: mol_type = genomic DNA
cttcaattatgatacatgaataaacaaaatattaaagaataaaattgtttttcttcattcatattgaatttttatttattattttgttaacttttgtcttttaaaaatttcaaagatatttcataaattcatctgaaattctcagatttataatgtaatgttgaaaaaatcgtatttatttttttgcgtaaatgaaagggaaattgatttcgcaatccaaaagaagaatttcttttacattttgtatttaaagatacgcaaaaaagaacacaaattcataataattttcaaagtcaacagaagtacattgcttctataaaaattatttaaaatttaaaatttgtgaaaagaattttaaaatgtgtggtagaaataaaaatcttaataaaagtcagtgcgagtgtcagcatcatcatcatcatcatttttatatcaatgaacagttaatagaacctgaggaaaaatcatcaaaattcaaatgattcagcaaaccatcaatacatcactatttttacttcaacgataagcaaataaataaagaagattgtcagccgaatgttgctacactcgcgaaaaatacagtaaaagaacatttcattcaacatcaaaaagctgcatctcaagaaaaaaattcaggctgctatcactttgaacataatccaattgataagaaatgggcacagtattttgaagagagatttggaaaatcacatggacatcaccattatcattcgttcaataatgatgattttccaaaaatgtttttcaacaaaaaatattttgaaggaagtttccttgattaagcaattcatatatttgaaagagaatttttgcatttgatttttttttcataaaaattaatttgtcgtttataaaacatatttgtcagtatgtttattttaaaaaatttaaatgagtaaaaaaactaatgaaaactataaataagtgaatttttatttcatttgtacaaacaatgattatcatcattatctcatcaatttcatcacttttagagaattttcacaaaaaaaaattatttttctacagaaaaatcacaaaataatgaaattcttatcaatataaaaaatgcatgtcattaccggcaattactcatatacaaaacaaacaagcacaaacacgttcaaaatcatattttcctcactatacaatataattattgtacacatgctcatttatttcacaagaattgtaaagaatattgtgagtgtatgtgaagcatataaaaagcagattaaatcgtacaacattcagttgacttatgatttctaaacgaataacatcgttggacaaaagaaaatattttctgaaaaaa

SEQ ID NO: 2 - protein, 454 aa, synthetic construct
MDAKDGEKEKAGEGMASMTGGQQMGRDLYDDDDKDLATMVDSSRRKWNKTGHAVRVIGRLSSLENVYIKADKQKNGIKANFHIRHNIEDGGVQLAYHYQQNTPIGDGPVLLPDNHYLSVQSKLSKDPNEKRDHMVLLEFVTAAGITLGMDELYKGGTGGSMVSKGEELFTGVVPILVELDGDVNGHKFSVSGEGEGDATYGKLTLKFICTTGKLPVPWPTLVTTLTYGVQCFSRYPDHMKQHDFFKSAMPEGYIQERTIFFKDDGNYKTRAEVKFEGDTLVNRIELKGIDFKEDGNILGHKLEYNLPDQLTEEQIAEFKELFSLFDKDGDGTITTKELGTVMRSLGQNPTEAELQDMINEVDADGDGTIDFPEFLTMMARKMKYRDTEEEIREAFGVFDKDGNGYISAAELRHVMTNLGEKLTDEEVDEMIREADIDGDGQVNYEEFVQMMTAK

SEQ ID NO: 3 - DNA, 1362 bp, synthetic construct
  source 1..1362: mol_type = other DNA
atggacgctaaggacggcgagaaagagaaggctggcgaaggcatggcttccatgaccggtggtcaacagatgggtcgtgacctgtacgacgacgatgacaaggacctggctaccatggtggactcctctcgtcgcaagtggaacaagaccggtcacgctgtgcgtgtgatcggtcgtctgtcctccttggagaacgtgtacatcaaggctgacaagcagaagaacggcatcaaggccaacttccacatccgtcacaacatcgaggacggtggtgtccagctggcttaccactaccagcagaacacccctatcggcgacggtcctgtgctgttgcctgacaaccactacctgtccgtgcagtccaagctgtctaaggaccccaacgagaagcgtgaccacatggtgctgctcgagttcgtgaccgctgctggtatcaccctcggaatggacgagctgtacaaaggtggcaccggtggttccatggtgtccaagggcgaagaactgttcaccggtgtcgtgcccatcctggtggaattggatggcgacgtgaacggtcacaagttctccgtttccggcgaaggcgagggcgacgctacttacggaaagctgaccctgaagttcatctgcaccaccggcaagctgcctgtgccttggcctactctggtcaccactctgacctacggtgtccagtgcttctctcgttaccccgaccatatgaagcagcacgacttcttcaagtccgctatgcccgagggttacatccaagagcgtaccattttcttcaaggacgacggcaactacaagacccgtgctgaagtgaagttcgaaggcgacaccctggtcaaccgtatcgagctgaagggtatcgacttcaaagaggacggaaacatcctgggtcacaagctcgagtacaacctgcctgaccagctgaccgaggaacagatcgctgagttcaaagagctgttctccctgttcgacaaagacggcgacggcaccatcaccaccaaagaactgggaaccgtgatgcgttccctgggacagaaccctactgaggctgagctgcaggacatgatcaacgaggtggacgctgatggcgacggtactatcgacttccccgagttcctgaccatgatggctcgcaagatgaagtaccgtgacactgaggaagagatccgcgaggctttcggtgttttcgacaaggatggcaacggttacatctccgctgccgagctgcgtcacgtgatgactaacctgggagagaagctgactgacgaagaggtcgacgagatgatccgtgaagctgacatcgacggcgacggtcaagtgaactacgaggaattcgtccagatgatgaccgccaag

SEQ ID NO: 4 - protein, 22 aa, synthetic construct
GSGATNFSLLKQAGDVEENPGP

SEQ ID NO: 5 - DNA, 66 bp, synthetic construct
  source 1..66: mol_type = other DNA
ggaagcggagctactaacttcagcctgctgaagcaggctggagacgtggaggagaaccctggacct

SEQ ID NO: 6 - protein, 21 aa, synthetic construct
GSGEGRGSLLTCGDVEENPGP

SEQ ID NO: 7 - DNA, 63 bp, synthetic construct
  source 1..63: mol_type = other DNA
ggaagcggagagggcagaggaagtctgctaacatgcggtgacgtcgaggagaatcctggacct

SEQ ID NO: 8 - protein, 199 aa, synthetic construct
MTEYKPTVRLATRDDVPRAVRTLAAAFADYPATRHTVDPDRHIERVTELQELFLTRVGLDIGKVWVADDGAAVAVWTTPESVEAGAVFAEIGPRMAELSGSRLAAQQQMEGLLAPHRPKEPAWFLATVGVSPDHQGKGLGSAVVLPGVEAAERAGVPAFLETSAPRNLPFYERLGFTVTADVEVPEGPRTWCMTRKPGA

SEQ ID NO: 9 - DNA, 597 bp, synthetic construct
  source 1..597: mol_type = other DNA
atgaccgagtacaagcccacggtgcgcctcgccacccgcgacgacgtccccagggccgtacgcaccctcgccgccgcgttcgccgactaccccgccacgcgccacaccgtcgatccggaccgccacatcgagcgggtcaccgagctgcaagaactcttcctcacgcgcgtcgggctcgacatcggcaaggtgtgggtcgcggacgacggcgccgcggtggcggtctggaccacgccggagagcgtcgaagcgggggcggtgttcgccgagatcggcccgcgcatggccgagttgagcggttcccggctggccgcgcagcaacagatggaaggcctcctggcgccgcaccggcccaaggagcccgcgtggttcctggccaccgtcggcgtctcgcccgaccaccagggcaagggtctgggcagcgccgtcgtgctccccggagtggaggcggccgagcgcgccggggtgcccgccttcctggagacatccgcgccccgcaacctccccttctacgagcggctcggcttcaccgtcaccgccgacgtcgaggtgcccgaaggaccgcgcacctggtgcatgacccgcaagcccggtgcc

SEQ ID NO: 10 - DNA, 230 bp, synthetic construct
  source 1..230: mol_type = other DNA
ctagatcataatcagccataccacatttgtagaggttttacttgctttaaaaaacctcccacacctccccctgaacctgaaacataaaatgaatgcaattgttgttgttaacttgtttattgcagcttataatggttacaaataaagcaatagcatcacaaatttcacaaataaagcatttttttcactgcattctagttgtggtttgtccaaactcatcaatgtatctt

SEQ ID NO: 11 - DNA, 1391 bp, Aedes aegypti
  source 1..1391: mol_type = genomic DNA
tatctttacatgtagcttgtgcattgaatccaattataatttgccttggcaccagctgagccagacaagaaagaaagcttcccagaagtatatcgatttagaagggttgacgtcacttgctgactgcactaatacagcaaatgatgcaattagaatgattcaagtgaaattcccaaattactgatttttctctggatttggttatcagattacattcgaagctaagattagctaccgaaattgtcgatcaaatcaggaaatcctttctctatcgaaaaaggcattcgcacatcttcctctctatgccatatacacgaagggtaggtacattgacgtctttgccagaagttgaactgcatcgttcaaggtacagaatgaacgactaacagacacaagcacgttttgctgtccattcagacacagggatggtacccatattcgatcgatatagagccatccaaccgaacagaggtatatgtatgaatgtattgctgaaattttctagaagtacaaccaccactacgacagtgtctataaaacgcccctgcaaaggcgaaaccagctcaatcgaatacgtttcctagtggagtgaacattacgcggcccaagtaagcagtgccagtgcaagtgaagtgaagtctctagtgaaaaagagtgatccaattagccagaggagaaaatttcagagtgaacaaagctttattcaaaggacaattactattaaattggtgaaagtgcatttcggtgaagggaatcttctagtgaaggtaggtaaattaattgatgaaattatagctatgagcgaaaactagtttggtgaatgattcctttgtctttgaatgagcaaactattttccaagatggcgactattgagctttgagtgattagtgaaaatttgcaacgcagtttcatcatcattgataaaacccaattgtgattcacagcgataatcatatttcgttgaatcatcgctactaattgaattaaatttctagaataataagaataacgtatttgctccgtcacatatctaaaataaatattttgatggtaattacccattaaggtaatattaacacatatcgagaaaaaccttgaggaaatcgtgaaaacttgaagatacgcaatttcaaaactacgtagttcaaagtcgaaaacaagttaatttttcacttaaaagtagggcgttgttgtgacgtcatcaccttcaagtgtatatttttcacttggcctgcgactgcaaacgcagacaaagcaaaacaagtttaaaacctgtcgtgtcgtgctcgaagccaaaggcaatgaatcaatatcaaatgagagtttgcatttcacaaccaattactcaagcgtttcctcgtttctttttctgctcaacagagatttcaac

SEQ ID NO: 12 - protein, 381 aa, Aedes aegypti
MESIIKLLKFCGFWGRPYQKFSLWQPLCHIAVLVVCLLAPGVIFIVRNSSNFASAISAAIESMGFINTILLGTTMLYHRSALENAYGDIRIALRIGKSSSIGDVQRNIEFLEKSTNFLFKGYTVFQSVVGTGYALTIPSLTVVYYVQTGQWPPLHGIFEADFFVFDFTTNVWLWVLVIAVGMFAMLCLISVLVIVSSFNWSFLHYIIGLFKLVHIRISRLNAFANPQSRQMELIEIVKLQELVYRCARTAEDTLNLFLLTQFGTCVVAICLTMMTLTLASNDQDLLIKMILMLAYILFNIFVYSMLGEELIATSTSLAEAAYGTQWYEWSIPEQRNILFIVRRSQKTAALTTGKFFAVNLAMFQAILSASYSYFTLLKDIF

SEQ ID NO: 13 - DNA, 1146 bp, Aedes aegypti
  source 1..1146: mol_type = genomic DNA
atggaatcgattatcaagttactaaaattctgcgggttctggggccgaccgtaccaaaagttcagcttgtggcaaccattgtgccacattgcagtgctcgtagtgtgcctcttggccccgggagtcatttttatcgttcgcaacagttcaaattttgcgagtgccattagtgctgccatcgaatcaatgggtttcattaatacgatcctgttgggaacaaccatgctgtatcatcgctctgccctggaaaacgcatacggagacattaggatcgctcttcggattggaaagtcctcgtcgattggggatgtgcaacggaatattgagtttttggaaaaatctacgaacttcctcttcaaaggatacacagtgtttcaatcggtggtgggaaccggatacgcactaaccattcctagtttgaccgtggtttactatgtgcaaactggccagtggcccccgctgcatggaatattcgaagcagatttcttcgtgtttgacttcaccacaaacgtctggctgtgggtgctggtgatcgccgttggaatgtttgcaatgctgtgtttaatctccgttctggtcatagtgagcagtttcaactggagtttcttgcattacatcatcggtttgttcaaactcgtgcacattagaatttctcgactgaacgccttcgcaaacccacaatcccgccagatggagctaatcgaaattgtcaaactgcaggaacttgtctacagatgtgcacggacggcggaagacaccctgaatctattcctgttgacgcaattcgggacgtgtgtcgttgccatttgcttgaccatgatgaccttaacattggcaagtaacgatcaagatttgctcatcaaaatgattctcatgttggcgtacattctgttcaacatatttgtctattccatgctgggagaggagctcatcgcaacgagtacatcattagcggaggccgcctacgggacgcaatggtatgaatggtcaatcccagagcagcgtaacatcttgttcattgtgaggagatcgcaaaagacagctgctcttaccacggggaaattcttcgccgttaatctagcgatgtttcaggcgattctttcagcgtcctattcgtactttaccctgctgaaggacatcttctga

SEQ ID NO: 14 - protein, 480 aa, synthetic construct
MTTSMQPSKYTGLVADLMPNIRAMKYSGLFMHNFTGGSAFMKKVYSSVHLVFLLMQFTFILVNMALNAEEVNELSGNTITTLFFTHCITKFIYLAVNQKNFYRTLNIWNQVNTHPLFAESDARYHSIALAKMRKLFFLVMLTTVASATAWTTITFFGDSVKMVVDHETNSSIPVEIPRLPIKSFYPWNASHGMFYMISFAFQIYYVLFSMIHSNLCDVMFCSWLIFACEQLQHLKNIMKPLMEFSATLDTVVPNSGELFKAGSAEQPKEQEPLPPVTPPQGENMLDMDLRGIYSNRTDFTTTFRPTAGMTFNGGVGPNGLTKKQEMLVRSAIKYWVERHKHIVRLVTAIGDAYGVALLLHMLTTTITLTLLAYQATKIHAVDTYAASVVGYLLYSLGQVFMLCIFGNRLIEESSSVMEAAYSCHWYDGSEEAKTFVQIVCQQCQKAMSISGAKFFTVSLDLFASVLGAMVTYFMVLVQLK

SEQ ID NO: 15 - DNA, 1443 bp, synthetic construct
  source 1..1443: mol_type = other DNA
atgacaacctcgatgcagccgagcaagtacacgggcctggtcgccgacctgatgcccaacatccgggcgatgaagtactccggcctgttcatgcacaacttcacgggcggcagtgccttcatgaagaaggtgtactcctccgtgcacctggtgttcctcctcatgcagttcaccttcatcctggtcaacatggccctgaacgccgaggaggtcaacgagctgtcgggcaacacgatcacgaccctcttcttcacccactgcatcacgaagtttatctacctggctgttaaccagaagaatttctacagaacattgaatatatggaaccaggtgaacacgcatcccttgttcgccgagtcggatgctcgttaccattcgatcgcactggcgaagatgaggaagctgttctttctggtgatgctgaccacagtcgcctcggccaccgcctggaccacgatcaccttctttggcgacagcgtaaaaatggtggtggaccatgagacgaactccagcatcccggtggagataccccggctgccgattaagtccttctacccgtggaacgccagccacggcatgttctacatgatcagctttgcctttcagatctactacgtgctcttctcgatgatccactccaatctatgcgacgtgatgttctgctcttggctgatattcgcctgcgagcagctgcagcacttgaagaatatcatgaagcctttgatggaattcagcgccacgctggacaccgtcgtgccaaacagtggggaactgttcaaggctggcagtgcagagcagccgaaggaacaggagccattgccaccagtcacgccgccccagggtgaaaacatgttggacatggatcttcgagggatatatagcaacaggaccgacttcacgaccaccttccggccaactgctggaatgacgttcaacggcggggtcgggccaaatgggttgaccaagaaacaggaaatgctggtacgaagcgccatcaagtactgggtagagagacacaagcatatcgttagactcgtaactgcaattggagacgcctatggtgtagctttgctgctacatatgttgactactactattacgttaactttgctcgcttaccaagcaacaaagatacatgcagtagatacatacgcagcatcagtagtaggttatttgctatattctttaggacaagtctttatgctctgtatatttggaaatcgtctcattgaagagagctcatcagtgatggaagcagcttattcttgtcactggtatgatggatcagaggaggccaaaacatttgtacagattgtttgccagcagtgtcagaaagcgatgtcgatttcaggggcaaagttcttcactgtatctttggatctctttgcttcggtgttgggagctatggttacctacttcatggtgttggtgcaactgaagtga